European Patent Specification EP 4 056 693 B1, published March 13, 2024. Title: Novel proline dehydrogenase variant and a method for producing L-valine using the same. Applicant: CJ CheilJedang Corporation. The sequence listing filed with the application follows.

SEQUENCE LISTING (11 sequences)

SEQ ID NO: 1 - protein, 1152 aa, Artificial Sequence
  Proline dehydrogenase variant
MTSMNLPIELATLSDQAVDKVRSWLEYSKKESVPNADAKRLAAVLQDPNGLEFTVGFVDRVVRTEDREAAAHALYELGKIAPSTMSFLDRAQIQAGSLVGRALPQVVVPAARARIRQMVGHMIVDARDKQFAKAVAEIQSDGHRLNINLLGEAVLGRKEAAKHLDDTVRLLRRPDVEYVSIKVSSVASQISMWGFEDTVTYVVEQLTPLYIEAARAPQGTKFINLDMEEYRDLRLTMEVFKRLLSKPELHELEAGIVLQAYLPDALGAIQDLAQFGRERVNTGGAGVKVRLVKGANLPMEHVHAQITGWPVATEPSKQATDANYKRVLYWTMRKENMEGLRLGVAGHNLFDIAFAHLLSVERGVADRVEFEMLQGMASDQARAVSVDVGELLLYVPAVRPQEFDVAISYLVRRLEENAASENFMSAIFDLDADNPSFKREESRFRASISDLATLIDVPAPGPNHTQDRSKETLLDAPLVPFINEPDTNPALIQNQQWATKALATAAEPGWLEKQTKPEVLEEGDVDKLINDVRDAAEAWAARPARERAEILYKTAEILRVRRGHLISVAAAEVGKAVEQTDPEISEAIDFARYYAHLALELDDVDNAEFTPDRVVVVTPPWNFPIAIPAGSTFAALAAGAGVIHKPSKPSQHCSAAVVEALWEAGVPREVLHCIYPANRDVGRALISHEHVDRVILTGSSETAAMFSSWRPELTINGETSGKNAIVVTPSADRDIAVADLVKSAFGHAGQKCSAASLGILVGSVYESERFRKQLVDAASSLIVDWPTNPSATVGPLTELPSDKLHHALTTLEEGESWLLKPRQLDDTGRLWSPSIKEGVKPGTFFHLTEVFGPVLGLMKATDLNEAIEFQNGNDFGLTGGLQSLDADEVRTWLDHVDVGNAYVNRGITGAIVQRQSFGGWKKSSVGLGSKAGGPNYVMLMGTWADAPSHHAPRKTNPLISKLDLSGEDIEWLEKANASDETAWNTEFGSPRDPSGLDVEANIFRYRPAEVVLRLDDSAIPRDAARVLLAARRAGVTPRVLQTPGVSEQVREVLSAAGVSAETVDDSVFISNVLRGEYDENSSVRVRYLGKVSDTVRERLAVRPEVVLLDDAVTASGRVELRYWLKEQAISMTLHRFGNPVAAFHELAEELKR

SEQ ID NO: 2 - DNA, 3459 bp, Artificial Sequence
  Proline dehydrogenase variant coding gene
atgacatcgatgaatctgcctattgagttggctacgctgtctgaccaggctgtggacaaggtgcgctcctggctggagtacagcaaaaaggaaagcgtgcccaatgccgatgcgaagcgtctagctgcagtgttgcaggatcctaatggtttggaattcacggttggtttcgtggatcgagtggttcgaactgaggatcgtgaagcggcagcgcatgcgttgtatgagttgggcaagattgctccgtcgacgatgtcctttttggatcgggcgcagattcaggctggttctttggtggggcgggcgttgccgcaggttgtggttcctgcggcgcgggctcgaatccggcagatggttgggcacatgattgtggatgcccgcgacaagcagttcgccaaggctgtcgctgagattcagtcggatgggcaccgcctgaacatcaatttgctaggtgaagcggtgttgggccgaaaggaggcagcgaagcatttggatgacacggtgcggttgttgcgccgtccggatgtggaatatgtgtccatcaaggtctcctcggtggcatcgcagatttcgatgtggggtttcgaagacaccgtcacttacgttgtggaacagctgacacctttatatatagaggccgcgcgggcgccccaaggcacgaagttcatcaacctggacatggaggaatatcgcgacctgcgtctgaccatggaagtgtttaaacggctgttgtccaagccggagctgcatgaactagaagccggaattgtgttgcaggcgtaccttcccgatgccctcggtgcgattcaggacctggcgcagttcggccgcgagcgcgtcaacacaggcggggcgggcgttaaggttcgcctggtcaagggggctaatttgcccatggagcacgtccatgcacagatcaccggctggccggttgctacggaaccttccaagcaagccactgatgccaactacaagcgcgtgctgtattggacgatgcgtaaagaaaacatggagggcctgcgcctgggtgttgccggccataaccttttcgacatagcattcgcgcatttactctctgtggagcgcggggttgccgaccgtgtggagttcgaaatgctgcagggcatggcgtccgatcaggcgcgcgccgtcagcgttgacgtcggtgagctgctgctttacgtaccagccgtgcgcccacaggaattcgacgtggccatttcttacctcgtgcgccgcctcgaggaaaacgccgcgagcgaaaacttcatgtccgccatcttcgacctcgacgccgacaacccgtccttcaagcgagaggagagccgcttccgcgcctccatatctgacctcgccacgcttatcgacgtgcccgcgcccggccccaaccacacacaagaccgcagcaaagagacgcttctcgacgcccccctcgtcccatttatcaacgagcccgacaccaacccagcgctcatccaaaaccaacagtgggccacaaaagccctcgccaccgcagcagagcccggttggttggaaaaacaaacaaagccggaggtgttggaagagggggacgtcgacaagctaattaacgatgtgcgcgacgctgctgaagcgtgggcagcgcgcccagcccgtgaacgcgctgagattttgtacaagaccgccgagattttgcgcgtgcgacgcggacacctgatctcagtggcggccgcggaggtgggcaaagctgtggaacaaaccgacccggaaatctctgaagccattgatttcgcccgctactacgcgcatttggccctggaattggacgacgtagacaatgcggaattcaccccagatcgcgtcgttgtggtgaccccgccctggaatttccccatcgcgatccccgctggatcgactttcgcagcactcgcggcgggcgctggcgtgatccacaaaccctcaaaacctagccaacattgctccgctgcagtggtcgaagccctctgggaagccggcgttccccgcgaggttctgcattgcatttacccagctaatcgcgatgttggacgtgcgttgatcagccatgaacacgtcgaccgcgtcattttgaccggctcctccgagaccgccgcgatgttctcctcctggcgaccagaactcaccatcaacggcgaaacctccggcaaaaacgccatcgtggtcaccccatctgccgaccgcgacatcgccgtcgccgacctggtgaaatccgccttcggccatgcaggacaaaaatgttccgcagcctccctcggcatcttggtaggcagcgtctacgaatcagaacgcttccggaaacagctggtagacgccgcatcctcactcatcgtcgactggcctaccaacccctccgcaaccgtcggaccactcaccgaactccccagcgataaactccaccacgccctaaccaccctcgaagaaggagaaagctggctgctgaaaccccgacaactcgacgacaccggccgactctggtcacccagcatcaaagaaggcgtcaaaccaggaaccttcttccacctcacagaagtattcggaccagtcctcggcctgatgaaagccaccgacctcaatgaagccatcgaattccaaaacggcaacgacttcggactcaccggcggactccaatccctcgacgccgacgaagtccgcacctggcttgaccacgtcgatgtcggaaacgcctacgtcaaccgcggcatcaccggcgccatcgtccaacgccaatccttcggaggctggaaaaaatcctccgtcggcctcggatccaaagccggaggacccaactatgtcatgctcatgggaacctgggccgacgcgccaagccaccacgccccacgcaaaacaaacccgctgatcagcaaactggatctgtccggtgaagacatcgaatggctcgaaaaagccaacgccagcgatgaaacagcatggaacacggaattcggcagcccacgcgacccctccggcctcgatgtagaagccaacatcttccgctaccgaccagcagaggtagtactccgactcgatgattccgctatacctcgcgatgctgcccgcgtacttttggcagcgcgccgcgccggggttactccgcgagttcttcaaacaccaggtgtttcagagcaagtccgcgaagtattgtccgctgctggagtgagtgcagaaacagtcgatgattcagtatttatttccaacgtgttgcgcggcgaatacgacgagaactccagcgtccgagtccgctacctgggcaaagttagcgacactgtccgtgaacgcctagctgtacggcccgaagttgttctgcttgacgatgcagtaactgcctccggtcgagttgaattacgttactggctcaaagaacaagcaatttccatgacgttgcaccgttttggaaacccagttgcggctttccacgagttggcggaggaacttaaacgttga

SEQ ID NO: 3 - protein, 1152 aa, Artificial Sequence
  Wild-type proline dehydrogenase
MTSMNLPIELATLSDQAVDKVRSWLEYSKKESVPNADAKRLAAVLQDPNGLEFTVGFVDRVVRTEDREAAAHALYELGKIAPSTMSFLDRAQIQAGSLVGRALPQVVVPAARARIRQMVGHMIVDARDKQFAKAVAEIQSDGHRLNINLLGEAVLGRKEAAKHLDDTVRLLRRPDVEYVSIKVSSVASQISMWGFEDTVTYVVEQLTPLYIEAARAPQGTKFINLDMEEYRDLRLTMEVFKRLLSKPELHELEAGIVLQAYLPDALGAIQDLAQFGRERVNTGGAGVKVRLVKGANLPMEHVHAQITGWPVATEPSKQATDANYKRVLYWTMRKENMEGLRLGVAGHNLFDIAFAHLLSVERGVADRVEFEMLQGMASDQARAVSVDVGELLLYVPAVRPQEFDVAISYLVRRLEENAASENFMSAIFDLDADNPSFKREESRFRASISDLATLIDVPAPGPNHTQDRSKETLLDAPLVPFINEPDTNPALIQNQQWATKALATAAEPGWLEKQTKPEVLEEGDVDKLINDVRDAAEAWAARPARERAEILYKTAEILRVRRGHLISVAAAEVGKAVEQTDPEISEAIDFARYYAHLALELDDVDNAEFTPDRVVVVTPPWNFPIAIPAGSTFAALAAGAGVIHKPSKPSQHCSAAVVEALWEAGVPREVLHCIYPANRDVGRALISHEHVDRVILTGSSETAAMFSSWRPELTINGETSGKNAIVVTPSADRDIAVADLVKSAFGHAGQKCSAASLGILVGSVYESERFRKQLVDAASSLIVDWPTNPSATVGPLTELPSDKLHHALTTLEEGESWLLKPRQLDDTGRLWSPGIKEGVKPGTFFHLTEVFGPVLGLMKATDLNEAIEFQNGNDFGLTGGLQSLDADEVRTWLDHVDVGNAYVNRGITGAIVQRQSFGGWKKSSVGLGSKAGGPNYVMLMGTWADAPSHHAPRKTNPLISKLDLSGEDIEWLEKANASDETAWNTEFGSPRDPSGLDVEANIFRYRPAEVVLRLDDSAIPRDAARVLLAARRAGVTPRVLQTPGVSEQVREVLSAAGVSAETVDDSVFISNVLRGEYDENSSVRVRYLGKVSDTVRERLAVRPEVVLLDDAVTASGRVELRYWLKEQAISMTLHRFGNPVAAFHELAEELKR

SEQ ID NO: 4 - DNA, 3459 bp, Artificial Sequence
  Wild-type proline dehydrogenase coding gene
atgacatcgatgaatctgcctattgagttggctacgctgtctgaccaggctgtggacaaggtgcgctcctggctggagtacagcaaaaaggaaagcgtgcccaatgccgatgcgaagcgtctagctgcagtgttgcaggatcctaatggtttggaattcacggttggtttcgtggatcgagtggttcgaactgaggatcgtgaagcggcagcgcatgcgttgtatgagttgggcaagattgctccgtcgacgatgtcctttttggatcgggcgcagattcaggctggttctttggtggggcgggcgttgccgcaggttgtggttcctgcggcgcgggctcgaatccggcagatggttgggcacatgattgtggatgcccgcgacaagcagttcgccaaggctgtcgctgagattcagtcggatgggcaccgcctgaacatcaatttgctaggtgaagcggtgttgggccgaaaggaggcagcgaagcatttggatgacacggtgcggttgttgcgccgtccggatgtggaatatgtgtccatcaaggtctcctcggtggcatcgcagatttcgatgtggggtttcgaagacaccgtcacttacgttgtggaacagctgacacctttatatatagaggccgcgcgggcgccccaaggcacgaagttcatcaacctggacatggaggaatatcgcgacctgcgtctgaccatggaagtgtttaaacggctgttgtccaagccggagctgcatgaactagaagccggaattgtgttgcaggcgtaccttcccgatgccctcggtgcgattcaggacctggcgcagttcggccgcgagcgcgtcaacacaggcggggcgggcgttaaggttcgcctggtcaagggggctaatttgcccatggagcacgtccatgcacagatcaccggctggccggttgctacggaaccttccaagcaagccactgatgccaactacaagcgcgtgctgtattggacgatgcgtaaagaaaacatggagggcctgcgcctgggtgttgccggccataaccttttcgacatagcattcgcgcatttactctctgtggagcgcggggttgccgaccgtgtggagttcgaaatgctgcagggcatggcgtccgatcaggcgcgcgccgtcagcgttgacgtcggtgagctgctgctttacgtaccagccgtgcgcccacaggaattcgacgtggccatttcttacctcgtgcgccgcctcgaggaaaacgccgcgagcgaaaacttcatgtccgccatcttcgacctcgacgccgacaacccgtccttcaagcgagaggagagccgcttccgcgcctccatatctgacctcgccacgcttatcgacgtgcccgcgcccggccccaaccacacacaagaccgcagcaaagagacgcttctcgacgcccccctcgtcccatttatcaacgagcccgacaccaacccagcgctcatccaaaaccaacagtgggccacaaaagccctcgccaccgcagcagagcccggttggttggaaaaacaaacaaagccggaggtgttggaagagggggacgtcgacaagctaattaacgatgtgcgcgacgctgctgaagcgtgggcagcgcgcccagcccgtgaacgcgctgagattttgtacaagaccgccgagattttgcgcgtgcgacgcggacacctgatctcagtggcggccgcggaggtgggcaaagctgtggaacaaaccgacccggaaatctctgaagccattgatttcgcccgctactacgcgcatttggccctggaattggacgacgtagacaatgcggaattcaccccagatcgcgtcgttgtggtgaccccgccctggaatttccccatcgcgatccccgctggatcgactttcgcagcactcgcggcgggcgctggcgtgatccacaaaccctcaaaacctagccaacattgctccgctgcagtggtcgaagccctctgggaagccggcgttccccgcgaggttctgcattgcatttacccagctaatcgcgatgttggacgtgcgttgatcagccatgaacacgtcgaccgcgtcattttgaccggctcctccgagaccgccgcgatgttctcctcctggcgaccagaactcaccatcaacggcgaaacctccggcaaaaacgccatcgtggtcaccccatctgccgaccgcgacatcgccgtcgccgacctggtgaaatccgccttcggccatgcaggacaaaaatgttccgcagcctccctcggcatcttggtaggcagcgtctacgaatcagaacgcttccggaaacagctggtagacgccgcatcctcactcatcgtcgactggcctaccaacccctccgcaaccgtcggaccactcaccgaactccccagcgataaactccaccacgccctaaccaccctcgaagaaggagaaagctggctgctgaaaccccgacaactcgacgacaccggccgactctggtcacccggcatcaaagaaggcgtcaaaccaggaaccttcttccacctcacagaagtattcggaccagtcctcggcctgatgaaagccaccgacctcaatgaagccatcgaattccaaaacggcaacgacttcggactcaccggcggactccaatccctcgacgccgacgaagtccgcacctggcttgaccacgtcgatgtcggaaacgcctacgtcaaccgcggcatcaccggcgccatcgtccaacgccaatccttcggaggctggaaaaaatcctccgtcggcctcggatccaaagccggaggacccaactatgtcatgctcatgggaacctgggccgacgcgccaagccaccacgccccacgcaaaacaaacccgctgatcagcaaactggatctgtccggtgaagacatcgaatggctcgaaaaagccaacgccagcgatgaaacagcatggaacacggaattcggcagcccacgcgacccctccggcctcgatgtagaagccaacatcttccgctaccgaccagcagaggtagtactccgactcgatgattccgctatacctcgcgatgctgcccgcgtacttttggcagcgcgccgcgccggggttactccgcgagttcttcaaacaccaggtgtttcagagcaagtccgcgaagtattgtccgctgctggagtgagtgcagaaacagtcgatgattcagtatttatttccaacgtgttgcgcggcgaatacgacgagaactccagcgtccgagtccgctacctgggcaaagttagcgacactgtccgtgaacgcctagctgtacggcccgaagttgttctgcttgacgatgcagtaactgcctccggtcgagttgaattacgttactggctcaaagaacaagcaatttccatgacgttgcaccgttttggaaacccagttgcggctttccacgagttggcggaggaacttaaacgttga

SEQ ID NO: 5 - DNA, 36 bp, Artificial Sequence
  putA_1F
tcgagctcggtacccccggcgttccccgcgaggttc

SEQ ID NO: 6 - DNA, 44 bp, Artificial Sequence
  putA_2R
ggtttgacgccttctttgatgctgggtgaccagagtcggccggt

SEQ ID NO: 7 - DNA, 44 bp, Artificial Sequence
  putA_3F
accggccgactctggtcacccagcatcaaagaaggcgtcaaacc

SEQ ID NO: 8 - DNA, 36 bp, Artificial Sequence
  putA_4R
ctctagaggatcccccggaagatgttggcttctaca

SEQ ID NO: 9 - DNA, 21 bp, Artificial Sequence
  putA_5F
ccggcgttccccgcgaggttc

SEQ ID NO: 10 - DNA, 21 bp, Artificial Sequence
  putA_6R
cggaagatgttggcttctaca

SEQ ID NO: 11 - DNA, 5803 bp, Artificial Sequence
  pDCM2
gttcgcttgctgtccataaaaccgcccagtctagctatcgccatgtaagcccactgcaagctacctgctttctctttgcgcttgcgttttcccttgtccagatagcccagtagctgacattcatccggggtcagcaccgtttctgcggactggctttctacgtgttccgcttcctttagcagcccttgcgccctgagtgcttgcggcagcgtgaagctagcttttatcgccattcgccattcaggctgcgcaactgttgggaagggcgatcggtgcgggcctcttcgctattacgccagctggcgaaagggggatgtgctgcaaggcgattaagttgggtaacgccagggttttcccagtcacgacgttgtaaaacgacggccagtgaattcgagctcggtacccggggatcctctagagtcgacctgcaggcatgcaagcttggcgtaatcatggtcatagctgtttcctgtgtgaaattgttatccgctcacaattccacacaacatacgagccggaagcataaagtgtaaagcctggggtgcctaatgagtgagctaactcacattaattgcgttgcgctcactgcccgctttccagtcgggaaacctgtcgtgccagctgcattaatgaatcggccaacgcgcggggagaggcggtttgcgtattgggcgctcttccgcttcctcgctcactgactcgctgcgctcggtcgttcggctgcggcgagcggtatcagctcactcaaaggcggtaatacggttatccacagaatcaggggataacgcaggaaagaacatgtgagcaaaaggccagcaaaaggccaggaaccgtaaaaaggccgcgttgctggcgtttttccataggctccgcccccctgacgagcatcacaaaaatcgacgctcaagtcagaggtggcgaaacccgacaggactataaagataccaggcgtttccccctggaagctccctcgtgcgctctcctgttccgaccctgccgcttaccggatacctgtccgcctttctcccttcgggaagcgtggcgctttctcaatgctcacgctgtaggtatctcagttcggtgtaggtcgttcgctccaagctgggctgtgtgcacgaaccccccgttcagcccgaccgctgcgccttatccggtaactatcgtcttgagtccaacccggtaagacacgacttatcgccactggcagcagccactggtaacaggattagcagagcgaggtatgtaggcggtgctacagagttcttgaagtggtggcctaactacggctacactagaaggacagtatttggtatctgcgctctgctgaagccagttaccttcggaaaaagagttggtagctcttgatccggcaaacaaaccaccgctggtagcggtggtttttttgtttgcaagcagcagattacgcgcagaaaaaaaggatctcaagaagatcctttgatcttttctacggggtctgacgctcagtggaacgaaaactcacgttaagggattttggtcatgagattatcaaaaaggatcttcacctagatccttttggggtgggcgaagaactccagcatgagatccccgcgctggaggatcatccagccctgatagaaacagaagccactggagcacctcaaaaacaccatcatacactaaatcagtaagttggcagcatcacccgacgcactttgcgccgaataaatacctgtgacggaagatcacttcgcagaataaataaatcctggtgtccctgttgataccgggaagccctgggccaacttttggcgaaaatgagacgttgatcggcacgtaagaggttccaactttcaccataatgaaataagatcactaccgggcgtattttttgagttatcgagattttcaggagctgatagaaacagaagccactggagcacctcaaaaacaccatcatacactaaatcagtaagttggcagcatcacccgacgcactttgcgccgaataaatacctgtgacggaagatcacttcgcagaataaataaatcctggtgtccctgttgataccgggaagccctgggccaacttttggcgaaaatgagacgttgatcggcacgtaagaggttccaactttcaccataatgaaataagatcactaccgggcgtattttttgagttatcgagattttcaggagctctttggcatcgtctctcgcctgtcccctcagttcagtaatttcctgcatttgcctgtttccagtcggtagatattccacaaaacagcagggaagcagcgcttttccgctgcataaccctgcttcggggtcattatagcgattttttcggtatatccatcctttttcgcacgatatacaggattttgccaaagggttcgtgtagactttccttggtgtatccaacggcgtcagccgggcaggataggtgaagtaggcccacccgcgagcgggtgttccttcttcactgtcccttattcgcacctggcggtgctcaacgggaatcctgctctgcgaggctggccggctaccgccggcgtaacagatgagggcaagcggatggctgatgaaaccaagccaaccaggaagggcagcccacctatcaaggtgtactgccttccagacgaacgaagagcgattgaggaaaaggcggcggcggccggcatgagcctgtcggcctacctgctggccgtcggccagggctacaaaatcacgggcgtcgtggactatgagcacgtccgcgagggcgtcccggaaaacgattccgaagcccaacctttcatagaaggcggcggtggaatcgaaatctcgtgatggcaggttgggcgtcgcttggtcggtcatttcgaaaaaggttaggaatacggttagccatttgcctgcttttatatagttcantatgggattcacctttatgttgataagaaataaaagaaaatgccaataggatatcggcattttcttttgcgtttttatttgttaactgttaattgtccttgttcaaggatgctgtctttgacaacagatgttttcttgcctttgatgttcagcaggaagctcggcgcaaacgttgattgtttgtctgcgtagaatcctctgtttgtcatatagcttgtaatcacgacattgtttcctttcgcttgaggtacagcgaagtgtgagtaagtaaaggttacatcgttaggcggatcaagatccatttttaacacaaggccagttttgttcagcggcttgtatgggccagttaaagaattagaaacataaccaagcatgtaaatatcgttagacgtaatgccgtcaatcgtcatttttgatccgcgggagtcagtgaacaggtaccatttgccgttcattttaaagacgttcgcgcgttcaatttcatctgttactgtgttagatgcaatcagcggtttcatcacttttttcagtgtgtaatcatcgtttagctcaatcataccgagagcgccgtttgctaactcagccgtgcgttttttatcgctttgcagaagtttttgactttcttgacggaagaatgatgtgcttttgccatagtatgctttgttaaataaagattcttcgccttggtagccatcttcagttccagtgtttgcttcaaatactaagtatttgtggcctttatcttctacgtagtgaggatctctcagcgtatggttgtcgcctgagctgtagttgccttcatcgatgaactgctgtacattttgatacgtttttccgtcaccgtcaaagattgatttataatcctctacaccgttgatgttcaaagagctgtctgatgctgatacgttaacttgtgcagttgtcagtgtttgtttgccgtaatgtttaccggagaaatcagtgtagaataaacggatttttccgtcagatgtaaatgtggctgaacctgaccattcttgtgtttggtcttttaggatagaatcatttgcatcgaatttgtcgctgtctttaaagacgcggccagcgtttttccagctgtcaatagaagtttcgccgactttttgatagaacatgtaaatcgatgtgtcatccgcatttttaggatctccggctaatgcaaagacgatgtggtagccgtgatagtttgcgacagtgccgtcagcgttttgtaatggccagctgtcccaaacgtccaggccttttgcagaagagatatttttaattgtggacgaatcaaattcagaaacttgatatttttcatttttttgctgttcagggatttgcagcatatcatggcgtgtaatatgggaaatgccgtatgtttccttatatggcttttggttcgtttctttcgcaaacgcttgagttgcgcctcctgccagcagtgcggtagtaaaggttaatactgttgcttgttttgcaaactttttgatgttcatcgttcatgtctccttttttatgtactgtgttagcggtctgcttcttccagccctcctgtttgaagatggcaagttagttacgcacaataaaaaaagacctaaaatatgtaaggggtgacgccaaagtatacactttgccctttacacattttaggtcttgcctgctttatcagtaacaaacccgcgcgatttacttttcgacctcattctattagactctcgtttggattgcaactggtctattttcctcttttgtttgatagaaaatcataaaaggatttgcagactacgggcctaaagaactaaaaaatctatctgtttcttttcattctctgtattttttatagtttctgttgcatgggcataaagttgcctttttaatcacaattcagaaaatatcataatatctcatttcactaaataatagtgaacggcaggtatatgtgatgggttaaaaaggatcaccccagagtcccgctcagaagaactcgtcaagaaggcgatagaaggcgatgcgctgcgaatcgggagcggcgataccgtaaagcacgaggaagcggtcagcccattcgccgccaagctcttcagcaatatcacgggtagccaacgctatgtcctgatagcggtccgccacacccagccggccacagtcgatgaatccagaaaagcggccattttccaccatgatattcggcaagcaggcatcgccatgggtcacgacgagatcctcgccgtcgggcatccgcgccttgagcctggcgaacagttcggctggcgcgagcccctgatgctcttcgtccagatcatcctgatcgacaagaccggcttccatccgagtacgtgctcgctcgatgcgatgtttcgcttggtggtcgaatgggcaggtagccggatcaagcgtatgcagccgccgcattgcatcagccatgatggatactttctcggcaggagcaaggtgagatgacaggagatcctgccccggcacttcgcccaatagcagccagtcccttcccgcttcagtgacaacgtcgagacagctgcgcaaggaacgcccgtcgtggccagccacgatagccgcgctgcctcgtcttggagttcattcagggcaccggacaggtcggtcttgacaaaaagaaccgggcgcccctgcgctgacagccggaacacggcggcatcagagcagccgattgtctgttgtgcccagtcatagccgaatagcctctccacccaagcggccggagaacctgcgtgcaatccatcttgttcaatcatgcgaaacgatcctcatcctgtctcttgatcagatcttgatcccctgcgccatcagatccttggcggcaagaaagccatccagtttactttgcagggcttcccaaccttaccagagggcgccccagctggcaattccg